European Patent Application EP 4 768 603 A1, published July 1, 2026. Title: METHOD OF DETECTING THE PRESENCE OF EXON 8 OF ANRIL IN A SUBJECT, KIT, SETS OF OLIGONUCLEOTIDES AND THEIR USES. Applicant: CNRS. Application EP. The sequence listing filed with the application follows.

SEQUENCE LISTING (11 sequences)

SEQ ID NO: 1 - DNA, 24 bp, synthetic construct
  source 1..24: mol_type = other DNA
tctatttggaatgtatctaactcc

SEQ ID NO: 2 - DNA, 21 bp, synthetic construct
  source 1..21: mol_type = other DNA
ttcatgctttggatatcagtg

SEQ ID NO: 3 - DNA, 42 bp, synthetic construct
  source 1..42: mol_type = other DNA
agttcaagaccagtctggccgaaaccatcagaggtaacagta

SEQ ID NO: 4 - DNA, 40 bp, synthetic construct
  source 1..40: mol_type = other DNA
caaagtgctgggattacaggtgaaggcgttcattggagag

SEQ ID NO: 5 - DNA, 21 bp, synthetic construct
  source 1..21: mol_type = other DNA
aacatggtgaaaccccgtctc

SEQ ID NO: 6 - DNA, 17 bp, synthetic construct
  source 1..17: mol_type = other DNA
accacacccggcggata

SEQ ID NO: 7 - RNA, 42 nt, synthetic construct
  source 1..42: mol_type = other RNA
taatttctactaagtgtagatacagtctctccaatgaacgcc

SEQ ID NO: 8 - DNA, 11 bp, synthetic construct
  source 1..11: mol_type = other DNA
ttattattatt

SEQ ID NO: 9 - RNA, 42 nt, synthetic construct
  source 1..42: mol_type = other RNA
ggtggcagcaagagaaaaatgaggaagaagcaaaagcggaaa

SEQ ID NO: 10 - RNA, 696 nt, Homo sapiens
  source 1..696: mol_type = genomic RNA
tctctccaatgaacgccttcactgatatccaaagcatgaaggacacaccagggaaaaacatagacctaacacaggacaaatggaattattagaaacattttctagcagaagaacactattctgttgccatttgaatctttgcttctttctaggtttgacaatgagcctatcatataagcccaaatgtaaacagaaagaggttgaatcagtcacgataagcccaattatgctgtggtaacaaacaacctcaaaatctcattggcttaaaatatacagaattattcttactcatggcacatatccatctatcatctgcaggggatctgctcactgaagtcacttaggaacttggactgatggaacggccactttttggtcactatatgtattaatctgttttaatcctgctgataaagacccaaaattgggaacaaaaagaagtttaactagacttacagttccgcatggctgaggaggcctcagaatcatggtgggaggcgaaaggcacttcttacatggtggcagcaagagaaaaatgaggaagaagcaaaagcggaaacctctgataaacccatcagatcttatgagacttattccactatcaagagaatagcatgggaaagactggctcccataatttacctccctctgggtccctccctcaacatgtgggaattctgggagaaacaattcaag

SEQ ID NO: 11 - RNA, 21 nt, synthetic construct
  source 1..21: mol_type = other RNA
taatttctactaagtgtagat